European Patent Application EP 4 620 479 A1, published September 24, 2025. Title: Postbiotic preparation for preventing or treating obesity. Applicant: Genbioma Aplicaciones S.L. The sequence listing filed with the application follows.

SEQUENCE LISTING (18 sequences)

SEQ ID NO: 1 - DNA, 20 bp, Mus musculus
  source 1..20: mol_type = other DNA
ctatgggatcagccagaaag

SEQ ID NO: 2 - DNA, 19 bp, Mus musculus
  source 1..19: mol_type = other DNA
agtcaaaggcatccaccaa

SEQ ID NO: 3 - DNA, 25 bp, Mus musculus
  source 1..25: mol_type = other DNA
cacagctgccttctgaaatgtgtgg

SEQ ID NO: 4 - DNA, 25 bp, Mus musculus
  source 1..25: mol_type = other DNA
tttctacgtggcccggttctaattc

SEQ ID NO: 5 - DNA, 19 bp, Mus musculus
  source 1..19: mol_type = other DNA
tctaggcaatgccgttcac

SEQ ID NO: 6 - DNA, 19 bp, Mus musculus
  source 1..19: mol_type = other DNA
gagcacatgggcaccatac

SEQ ID NO: 7 - DNA, 21 bp, Mus musculus
  source 1..21: mol_type = other DNA
agccatggaggaggtggtgat

SEQ ID NO: 8 - DNA, 21 bp, Mus musculus
  source 1..21: mol_type = other DNA
gtgtgcctgcttggggtggac

SEQ ID NO: 9 - DNA, 21 bp, Mus musculus
  source 1..21: mol_type = other DNA
aaagccgctcgcaagagtgcg

SEQ ID NO: 10 - DNA, 20 bp, Mus musculus
  source 1..20: mol_type = other DNA
acttgcctcctgcaaagcac

SEQ ID NO: 11 - DNA, 19 bp, Mus musculus
  source 1..19: mol_type = genomic DNA
acaaggcctcagggtacca

SEQ ID NO: 12 - DNA, 20 bp, Mus musculus
  source 1..20: mol_type = other DNA
gccgaaagaagcccttacag

SEQ ID NO: 13 - DNA, 21 bp, Mus musculus
  source 1..21: mol_type = other DNA
gctgttatgggtgaaactctg

SEQ ID NO: 14 - DNA, 23 bp, Mus musculus
  source 1..23: mol_type = other DNA
gaataataaggtggagatgcagg

SEQ ID NO: 15 - DNA, 20 bp, Mus musculus
  source 1..20: mol_type = other DNA
agtcatcatcacccaagagc

SEQ ID NO: 16 - DNA, 19 bp, Mus musculus
  source 1..19: mol_type = other DNA
gggatgacatacatggtgc

SEQ ID NO: 17 - DNA, 20 bp, Mus musculus
  source 1..20: mol_type = other DNA
cacttcatcaaggcagactc

SEQ ID NO: 18 - DNA, 20 bp, Mus musculus
  source 1..20: mol_type = other DNA
cggtagcgcttctcaatggc